European Patent Application EP 4 239 061 A1, published September 6, 2023. Title: Method for the generation of outer radial glial (oRG) cells. Applicant: Max-Planck-Gesellschaft zur Förderung der Wissenschaften e.V. The sequence listing filed with the application follows.

SEQUENCE LISTING (22 sequences)

SEQ ID NO: 1 - protein, 213 aa, Mus musculus
  Mouse Noggin (Leu20Cys232)
LRAAPAGGQHYLHIRPAPSDNLPLVDLIEHPDPIFDPKEKDLNETLLRSLLGGHYDPGFMATSPPEDRPGGGGGPAGGAEDLAELDQLLRQRPSGAMPSEIKGLEFSEGLAQGKKQRLSKKLRRKLQMWLWSQTFCPVLYAWNDLGSRFWPRYVKVGSCFSKRSCSVPEGMVCKPSKSVHLTVLRWRCQRRGGQRCGWIPIQYPIISECKCSC

SEQ ID NO: 2 - protein, 6 aa, Artificial Sequence
  polypeptide linker
IEGRMD

SEQ ID NO: 3 - protein, 231 aa, Homo sapiens
  Human IgG1 (Pro100-Lys330)
PKSCDKTHTCPPCPAPELLGGPSVFLFPPKPKDTLMISRTPEVTCVVVDVSHEDPEVKFNWYVDGVEVHNAKTKPREEQYNSTYRVVSVLTVLHQDWLNGKEYKCKVSNKALPAPIEKTISKAKGQPREPQVYTLPPSRDELTKNQVSLTCLVKGFYPSDIAVEWESNGQPENNYKTTPPVLDSDGSFFLYSKLTVDKSRWQQGNVFSCSVMHEALHNHYTQKSLSLSPGK

SEQ ID NO: 4 - protein, 450 aa, Artificial Sequence
  Mouse Noggin + polypeptide linker + Fc region of human IgG1
LRAAPAGGQHYLHIRPAPSDNLPLVDLIEHPDPIFDPKEKDLNETLLRSLLGGHYDPGFMATSPPEDRPGGGGGPAGGAEDLAELDQLLRQRPSGAMPSEIKGLEFSEGLAQGKKQRLSKKLRRKLQMWLWSQTFCPVLYAWNDLGSRFWPRYVKVGSCFSKRSCSVPEGMVCKPSKSVHLTVLRWRCQRRGGQRCGWIPIQYPIISECKCSCIEGRMDPKSCDKTHTCPPCPAPELLGGPSVFLFPPKPKDTLMISRTPEVTCVVVDVSHEDPEVKFNWYVDGVEVHNAKTKPREEQYNSTYRVVSVLTVLHQDWLNGKEYKCKVSNKALPAPIEKTISKAKGQPREPQVYTLPPSRDELTKNQVSLTCLVKGFYPSDIAVEWESNGQPENNYKTTPPVLDSDGSFFLYSKLTVDKSRWQQGNVFSCSVMHEALHNHYTQKSLSLSPGK

SEQ ID NO: 5 - RNA, 23 nt, Homo sapiens
  miR20b sequence
caaagugcucauagugcagguag

SEQ ID NO: 6 - DNA, 23 bp, Homo sapiens
  miR20b complementary sequence
ctaactgcactagatgcacctta

SEQ ID NO: 7 - DNA, 142 bp, Artificial Sequence
  /note="combined DNA/RNA molecule" /note="miR20b construct"
gaaggctcgagaaggtatattgctgttgacagtgagcgcaaagugcucauagugcagguagctgtgaagccacagatgggctaactgcactagatgcaccttatgcctactgcctcggacttcaaggggctagaattcgagc

SEQ ID NO: 8 - protein, 4 aa, Artificial Sequence
  Thioredoxin-A variable peptide loop
CGPC

SEQ ID NO: 9 - DNA, 20 bp, Artificial Sequence
  BRACHYURY Forward
acccagttcatagcggtgac

SEQ ID NO: 10 - DNA, 20 bp, Artificial Sequence
  BRACHYURY Reverse
caattgtcatgggattgcag

SEQ ID NO: 11 - DNA, 21 bp, Artificial Sequence
  FOXA2 Forward
ccgactggagcagctactatg

SEQ ID NO: 12 - DNA, 20 bp, Artificial Sequence
  FOXA2 Reverse
tgtacgtgttcatgccgttc

SEQ ID NO: 13 - DNA, 21 bp, Artificial Sequence
  HPRT Forward
tgacactggcaaaacaatgca

SEQ ID NO: 14 - DNA, 21 bp, Artificial Sequence
  HPRT Reverse
ggtccttttcaccagcaagct

SEQ ID NO: 15 - DNA, 18 bp, Artificial Sequence
  OCT4 Forward
cagcagatcagccacatc

SEQ ID NO: 16 - DNA, 19 bp, Artificial Sequence
  OCT4 Reverse
cggttacagaaccacactc

SEQ ID NO: 17 - DNA, 20 bp, Artificial Sequence
  SOX1 Forward
gcaagatggcccaggagaac

SEQ ID NO: 18 - DNA, 20 bp, Artificial Sequence
  SOX1 Reverse
cggacatgaccttccactcg

SEQ ID NO: 19 - DNA, 19 bp, Artificial Sequence
  SOX17 Forward
aagatgactggcaagtcgt

SEQ ID NO: 20 - DNA, 18 bp, Artificial Sequence
  SOX17 Reverse
cttcagccgcttcacctg

SEQ ID NO: 21 - DNA, 20 bp, Artificial Sequence
  SOX2 Forward
gcaagatggcccaggagaac

SEQ ID NO: 22 - DNA, 21 bp, Artificial Sequence
  SOX2 Reverse
ccgacaaaagtttccactcgg